European Patent Specification EP 3 669 001 B1, published July 17, 2024. Title: Amplicon region as epigenetic marker for the identification of immune cells, in particular non-classical monocytes. Applicant: Epiontis GmbH. The sequence listing filed with the application follows.

SEQUENCE LISTING (11 sequences)

SEQ ID NO: 1 - DNA, 271 bp, Homo sapiens
cccttcctctgactcagtggaagggcaggagagtgccccgaggagctgcccacatccctggctgagtgcctcacccccagggcctccacgaggagcagcttccacagggtgcctgtggggctcgttcctctggatgcttttccctttgctgtgaatgcctctggggcacgaatatatggcccttgggtctaggccttagggcttccggtgaccaggataggaagtgttgcaggccctgccccgagggcggcgcattagcttttcccccact

SEQ ID NO: 2 - DNA, 300 bp, Homo sapiens
cccttcctctaactcaataaaaaaacaaaaaaataccccaaaaaactacccacatccctaactaaatacctcacccccaaaacctccacaaaaaacaacttccacaaaatacctataaaactcattcctctaaatacttttccctttactataaatacctctaaaacacaaatatataacccttaaatctaaaccttaaaacttccaataaccaaaataaaaaatattacaaaccctaccccaaaaacaacacattaacttttcccccactactttcatctacccatctcaccaaattcc

SEQ ID NO: 3 - DNA, 300 bp, Homo sapiens
cccttcctctaactcaataaaaaaacaaaaaaataccccgaaaaactacccacatccctaactaaatacctcacccccaaaacctccacgaaaaacaacttccacaaaatacctataaaactcgttcctctaaatacttttccctttactataaatacctctaaaacacgaatatataacccttaaatctaaaccttaaaacttccgataaccaaaataaaaaatattacaaaccctaccccgaaaacgacgcattaacttttcccccactactttcatctacccatctcaccaaattcc

SEQ ID NO: 4 - DNA, 22 bp, Homo sapiens
cccttcctctaactcaataaaa

SEQ ID NO: 5 - DNA, 19 bp, Homo sapiens
agtgggggaaaagttaatg

SEQ ID NO: 6 - DNA, 29 bp, Homo sapiens
cccttaaatctaaaccttaaaacttccaa

SEQ ID NO: 7 - DNA, 24 bp, Homo sapiens
tagtgggggaaaagttaatgtgtt

SEQ ID NO: 8 - DNA, 25 bp, Homo sapiens
acaaaccctaccccaaaaacaacac

SEQ ID NO: 9 - DNA, 28 bp, Homo sapiens
ccttaaatctaaaccttaaaacttccga

SEQ ID NO: 10 - DNA, 22 bp, Homo sapiens
gtggaggaaaagttaatgcgtc

SEQ ID NO: 11 - DNA, 24 bp, Homo sapiens
caaaccctaccccgaaaacgacgc